European Patent Specification EP 4 118 197 B1, published October 23, 2024. Title: HIGH FIDELITY SPCAS9 NUCLEASES FOR GENOME MODIFICATION. Applicant: SIGMA-ALDRICH CO. LLC. The sequence listing filed with the application follows.

SEQUENCE LISTING (83 sequences)

SEQ ID NO: 1 - protein, 1368 aa, Streptococcus pyogenes [sequence omitted]

SEQ ID NO: 2 - protein, 7 aa, Artificial Sequence
  source: /note="Description of Artificial Sequence: Synthetic peptide"
PKKKRKV

SEQ ID NO: 3 - protein, 7 aa, Artificial Sequence
  source: /note="Description of Artificial Sequence: Synthetic peptide"
PKKKRRV

SEQ ID NO: 4 - protein, 16 aa, Artificial Sequence
  source: /note="Description of Artificial Sequence: Synthetic peptide"
KRPAATKKAGQAKKKK

SEQ ID NO: 5 - protein, 11 aa, Artificial Sequence
  source: /note="Description of Artificial Sequence: Synthetic peptide"
YGRKKRRQRRR

SEQ ID NO: 6 - protein, 9 aa, Artificial Sequence
  source: /note="Description of Artificial Sequence: Synthetic peptide"
RKKRRQRRR

SEQ ID NO: 7 - protein, 9 aa, Artificial Sequence
  source: /note="Description of Artificial Sequence: Synthetic peptide"
PAAKRVKLD

SEQ ID NO: 8 - protein, 11 aa, Artificial Sequence
  source: /note="Description of Artificial Sequence: Synthetic peptide"
RQRRNELKRSP

SEQ ID NO: 9 - protein, 8 aa, Artificial Sequence
  source: /note="Description of Artificial Sequence: Synthetic peptide"
VSRKRPRP

SEQ ID NO: 10 - protein, 8 aa, Artificial Sequence
  source: /note="Description of Artificial Sequence: Synthetic peptide"
PPKKARED

SEQ ID NO: 11 - protein, 8 aa, Artificial Sequence
  source: /note="Description of Artificial Sequence: Synthetic peptide"
PQPKKKPL

SEQ ID NO: 12 - protein, 12 aa, Artificial Sequence
  source: /note="Description of Artificial Sequence: Synthetic peptide"
SALIKKKKKMAP

SEQ ID NO: 13 - protein, 7 aa, Artificial Sequence
  source: /note="Description of Artificial Sequence: Synthetic peptide"
PKQKKRK

SEQ ID NO: 14 - protein, 10 aa, Artificial Sequence
  source: /note="Description of Artificial Sequence: Synthetic peptide"
RKLKKKIKKL

SEQ ID NO: 15 - protein, 10 aa, Artificial Sequence
  source: /note="Description of Artificial Sequence: Synthetic peptide"
REKKKFLKRR

SEQ ID NO: 16 - protein, 20 aa, Artificial Sequence
  source: /note="Description of Artificial Sequence: Synthetic peptide"
KRKGDEVDGVDEVAKKKSKK

SEQ ID NO: 17 - protein, 17 aa, Artificial Sequence
  source: /note="Description of Artificial Sequence: Synthetic peptide"
RKCLQAGMNLEARKTKK

SEQ ID NO: 18 - protein, 38 aa, Artificial Sequence
  source: /note="Description of Artificial Sequence: Synthetic polypeptide"
NQSSNFGPMKGGNFGGRSSGPYGGGGQYFAKPRNQGGY

SEQ ID NO: 19 - protein, 42 aa, Artificial Sequence
  source: /note="Description of Artificial Sequence: Synthetic polypeptide"
RMRIZFKNKGKDTAELRRRRVEVSVELRKAKKDEQILKRRNV

SEQ ID NO: 20 - protein, 20 aa, Artificial Sequence
  source: /note="Description of Artificial Sequence: Synthetic peptide"
GRKKRRQRRRPPQPKKKRKV

SEQ ID NO: 21 - protein, 19 aa, Artificial Sequence
  source: /note="Description of Artificial Sequence: Synthetic peptide"
PLSSIFSRIGDPPKKKRKV

SEQ ID NO: 22 - protein, 24 aa, Artificial Sequence
  source: /note="Description of Artificial Sequence: Synthetic peptide"
GALFLGWLGAAGSTMGAPKKKRKV

SEQ ID NO: 23 - protein, 27 aa, Artificial Sequence
  source: /note="Description of Artificial Sequence: Synthetic peptide"
GALFLGFLGAAGSTMGAWSQPKKKRKV

SEQ ID NO: 24 - protein, 21 aa, Artificial Sequence
  source: /note="Description of Artificial Sequence: Synthetic peptide"
KETWWETWWTEWSQPKKKRKV

SEQ ID NO: 25 - protein, 11 aa, Artificial Sequence
  source: /note="Description of Artificial Sequence: Synthetic peptide"
YARAAARQARA

SEQ ID NO: 26 - protein, 11 aa, Artificial Sequence
  source: /note="Description of Artificial Sequence: Synthetic peptide"
THRLPRRRRRR

SEQ ID NO: 27 - protein, 11 aa, Artificial Sequence
  source: /note="Description of Artificial Sequence: Synthetic peptide"
GGRRARRRRRR

SEQ ID NO: 28 - protein, 12 aa, Artificial Sequence
  source: /note="Description of Artificial Sequence: Synthetic peptide"
RRQRRTSKLMKR

SEQ ID NO: 29 - protein, 27 aa, Artificial Sequence
  source: /note="Description of Artificial Sequence: Synthetic peptide"
GWTLNSAGYLLGKINLKALAALAKKIL

SEQ ID NO: 30 - protein, 33 aa, Artificial Sequence
  source: /note="Description of Artificial Sequence: Synthetic polypeptide"
KALAWEAKLAKALAKALAKHLAKALAKALKCEA

SEQ ID NO: 31 - protein, 16 aa, Artificial Sequence
  source: /note="Description of Artificial Sequence: Synthetic peptide"
RQIKIWFQNRRMKWKK

SEQ ID NO: 32 - protein, 6 aa, Artificial Sequence
  source: /note="Description of Artificial Sequence: Synthetic 6xHis tag"
HHHHHH

SEQ ID NO: 33 - protein, 6 aa, Artificial Sequence
  source: /note="Description of Artificial Sequence: Synthetic peptide"
LEGGGS

SEQ ID NO: 34 - protein, 4 aa, Artificial Sequence
  source: /note="Description of Artificial Sequence: Synthetic peptide"
TGSG

SEQ ID NO: 35 - protein, 8 aa, Artificial Sequence
  source: /note="Description of Artificial Sequence: Synthetic peptide"
GGSGGGSG

SEQ ID NO: 36 - protein, 20 aa, Artificial Sequence
  source: /note="Description of Artificial Sequence: Synthetic peptide"
  SITE (1)..(20): /note="This sequence may encompass 1-4 'Gly Gly Gly Gly Ser' repeating units"
GGGGSGGGGSGGGGSGGGGS

SEQ ID NO: 37 - protein, 8 aa, Artificial Sequence
  source: /note="Description of Artificial Sequence: Synthetic peptide"
  SITE (1)..(8): /note="This sequence may encompass 6-8 residues"
GGGGGGGG

SEQ ID NO: 38 - protein, 20 aa, Artificial Sequence
  source: /note="Description of Artificial Sequence: Synthetic peptide"
  SITE (1)..(20): /note="This sequence may encompass 1-4 'Glu Ala Ala Ala Lys' repeating units"
EAAAKEAAAKEAAAKEAAAK

SEQ ID NO: 39 - protein, 27 aa, Artificial Sequence
  source: /note="Description of Artificial Sequence: Synthetic peptide"
  SITE (2)..(26): /note="This region may encompass 2-5 'Glu Ala Ala Ala Lys' repeating units"
AEAAAKEAAAKEAAAKEAAAKEAAAKA

SEQ ID NO: 40 - protein, 5 aa, Artificial Sequence
  source: /note="Description of Artificial Sequence: Synthetic peptide"
PAPAP

SEQ ID NO: 41 - protein, 16 aa, Artificial Sequence
  source: /note="Description of Artificial Sequence: Synthetic peptide"
  SITE (1)..(16): /note="This sequence may encompass 6-8 'Ala Pro' repeating units"
APAPAPAPAPAPAPAP

SEQ ID NO: 42 - RNA, 20 nt, Artificial Sequence
  source: /note="Description of Artificial Sequence: Synthetic oligonucleotide"
ggcacugcggcuggaggugg

SEQ ID NO: 43 - DNA, 59 bp, Artificial Sequence
  source: /note="Description of Artificial Sequence: Synthetic primer"
  modified_base (34)..(39): a, c, t, g, unknown or other
tcgtcggcagcgtcagatgtgtataagagacagnnnnnnggaacccaggtagccagaga

SEQ ID NO: 44 - DNA, 57 bp, Artificial Sequence
  source: /note="Description of Artificial Sequence: Synthetic primer"
  modified_base (35)..(40): a, c, t, g, unknown or other
gtctcgtgggctcggagatgtgtataagagacagnnnnnnggggtggggtcagacgt

SEQ ID NO: 45 - DNA, 63 bp, Artificial Sequence
  source: /note="Description of Artificial Sequence: Synthetic primer"
  modified_base (34)..(39): a, c, t, g, unknown or other
tcgtcggcagcgtcagatgtgtataagagacagnnnnnnctagagcaaaccttggcattgtcc

SEQ ID NO: 46 - DNA, 60 bp, Artificial Sequence
  source: /note="Description of Artificial Sequence: Synthetic primer"
  modified_base (35)..(40): a, c, t, g, unknown or other
gtctcgtgggctcggagatgtgtataagagacagnnnnnnaccctctaccctccctgatg

SEQ ID NO: 47 - protein, 1404 aa, Artificial Sequence
  source: /note="Description of Artificial Sequence: Synthetic polypeptide"
PAAKRVKLDGGGGSTGMDKKYSIGLDIGTNSVGWAVITDEYKVPSKKFKVLGTDRHSIKKNLIGALLFDSGETAEATRLKRTARRRYTRRKNRICYLQEIFSNEMAKVDDSFFHRLEESFLVEEDKKHERHPIFGNIVDEVAYHEKYPTIYHLRKKLVDSTDKADLRLIYLALAHMIKFRGHFLIEGDLNPDNSDVDKLFIQLVQTYNQLFEENPINASGVDAKAILSARLSKSRRLENLIAQLPGEKKNGLFGNLIALSLGLTPNFKSNFDLAEDAKLQLSKDTYDDDLDNLLAQIGDQYADLFLAAKNLSDAILLSDILRVNTEITKAPLSASMIKRYDEHHQDLTLLKALVRQQLPEKYKEIFFDQSKNGYAGYIDGGASQEEFYKFIKPILEKMDGTEELLVKLNREDLLRKQRTFDNGSIPHQIHLGELHAILRRQEDFYPFLKDNREKIEKILTFRIPYYVGPLARGNSRFAWMTRKSEETITPWNFEEVVDKGASAQSFIERMTNFDKNLPNEKVLPKHSLLYEYFTVYNELTKVKYVTEGMRKPAFLSGEQKKAIVDLLFKTNRKVTVKQLKEDYFKKIECFDSVEISGVEDRFNASLGTYHDLLKIIKDKDFLDNEENEDILEDIVLTLTLFEDREMIEERLKTYAHLFDDKVMKQLKRRRYTGWGRLSRKLINGIRDKQSGKTILDFLKSDGFANRNFMQLIHDDSLTFKEDIQKAQVSGQGDSLHEHIANLAGSPAIKKGILQTVKVVDELVKVMGRHKPENIVIEMARENQTTQKGQKNSRERMKRIEEGIKELGSQILKEHPVENTQLQNEKLYLYYLQNGRDMYVDQELDINRLSDYDVDHIVPQSFLKDDSIDNQVLTRSDKNRGKSDNVPSEEVVKKMKNYWRQLLNAKLITQRKFDNLTKAERGGLSELDKAGFIKRQLVETRQITKHVAQILDSRMNTKYDENDKLIREVKVITLKSKLVSDFRKDFQFYKVREINNYHHAHDAYLNAVVGTALIKKYPKLESEFVYGDYKVYDVRKMIAKSEQEIGKATAKYFFYSNIMNFFKTEITLANGEIRKRPLIETNGETGEIVWDKGRDFATVRKVLSMPQVNIVKKTEVQTGGFSKESILPKRNSDKLIARKKDWDPKKYGGFDSPTVAYSVLVVAKVEKGKSKKLKSVKELLGITIMERSSFEKNPIDFLEAKGYKEVKKDLIIKLPKYSLFELENGRKRMLASAGELQKGNELALPSKYVNFLYLASHYEKLKGSPEDNEQKQLFVEQHKHYLDEIIEQISEFSKRVILADANLDKVLSAYNKHRDKPIREQAENIIHLFTLTNLGAPAAFKYFDTTIDRKRYTSTKEVLDATLIHQSITGLYETRIDLSQLGGDEFPKKKRKVGGGGSPKKKRKV

SEQ ID NO: 48 - RNA, 20 nt, Artificial Sequence
  source: /note="Description of Artificial Sequence: Synthetic oligonucleotide"
gcugcagaagggauuccaug

SEQ ID NO: 49 - RNA, 20 nt, Artificial Sequence
  source: /note="Description of Artificial Sequence: Synthetic oligonucleotide"
cacguucaccuugccccaca

SEQ ID NO: 50 - DNA, 59 bp, Artificial Sequence
  source: /note="Description of Artificial Sequence: Synthetic primer"
  modified_base (34)..(39): a, c, t, g, unknown or other
tcgtcggcagcgtcagatgtgtataagagacagnnnnnnaatggggccatgccgaccaa

SEQ ID NO: 51 - DNA, 63 bp, Artificial Sequence
  source: /note="Description of Artificial Sequence: Synthetic primer"
  modified_base (35)..(40): a, c, t, g, unknown or other
gtctcgtgggctcggagatgtgtataagagacagnnnnnnagttgcccagagtcaaggaacac

SEQ ID NO: 52 - DNA, 60 bp, Artificial Sequence
  source: /note="Description of Artificial Sequence: Synthetic primer"
  modified_base (34)..(39): a, c, t, g, unknown or other
tcgtcggcagcgtcagatgtgtataagagacagnnnnnntctttccctcactctggctcg

SEQ ID NO: 53 - DNA, 61 bp, Artificial Sequence
  source: /note="Description of Artificial Sequence: Synthetic primer"
  modified_base (35)..(40): a, c, t, g, unknown or other
gtctcgtgggctcggagatgtgtataagagacagnnnnnntggaatgaatggggtgggagg

SEQ ID NO: 54 - DNA, 63 bp, Artificial Sequence
  source: /note="Description of Artificial Sequence: Synthetic primer"
  modified_base (34)..(39): a, c, t, g, unknown or other
tcgtcggcagcgtcagatgtgtataagagacagnnnnnntaggcagagagagtcagtgcctat

SEQ ID NO: 55 - DNA, 61 bp, Artificial Sequence
  source: /note="Description of Artificial Sequence: Synthetic primer"
  modified_base (35)..(40): a, c, t, g, unknown or other
gtctcgtgggctcggagatgtgtataagagacagnnnnnnccaatctactcccaggagcag

SEQ ID NO: 56 - DNA, 59 bp, Artificial Sequence
  source: /note="Description of Artificial Sequence: Synthetic primer"
  modified_base (34)..(39): a, c, t, g, unknown or other
tcgtcggcagcgtcagatgtgtataagagacagnnnnnntcactggagcagggaggaca

SEQ ID NO: 57 - DNA, 61 bp, Artificial Sequence
  source: /note="Description of Artificial Sequence: Synthetic primer"
  modified_base (35)..(40): a, c, t, g, unknown or other
gtctcgtgggctcggagatgtgtataagagacagnnnnnngggtaggaaaacagcccaagg

SEQ ID NO: 58 - RNA, 20 nt, Artificial Sequence
  source: /note="Description of Artificial Sequence: Synthetic oligonucleotide"
cucccucccaggauccucuc

SEQ ID NO: 59 - RNA, 20 nt, Artificial Sequence
  source: /note="Description of Artificial Sequence: Synthetic oligonucleotide"
gccaguagccagccccgucc

SEQ ID NO: 60 - RNA, 20 nt, Artificial Sequence
  source: /note="Description of Artificial Sequence: Synthetic oligonucleotide"
caggcagucuucauccccgu

SEQ ID NO: 61 - RNA, 20 nt, Artificial Sequence
  source: /note="Description of Artificial Sequence: Synthetic oligonucleotide"
gaagcgugaugacaaagagg

SEQ ID NO: 62 - RNA, 20 nt, Artificial Sequence
  source: /note="Description of Artificial Sequence: Synthetic oligonucleotide"
auucuggucaacguguccuu

SEQ ID NO: 63 - DNA, 62 bp, Artificial Sequence
  source: /note="Description of Artificial Sequence: Synthetic primer"
  modified_base (34)..(39): a, c, t, g, unknown or other
tcgtcggcagcgtcagatgtgtataagagacagnnnnnncttgggaagtgtaaggaagctgc

SEQ ID NO: 64 - DNA, 61 bp, Artificial Sequence
  source: /note="Description of Artificial Sequence: Synthetic primer"
  modified_base (35)..(40): a, c, t, g, unknown or other
gtctcgtgggctcggagatgtgtataagagacagnnnnnngcctcctccttcctagtctcc

SEQ ID NO: 65 - DNA, 61 bp, Artificial Sequence
  source: /note="Description of Artificial Sequence: Synthetic primer"
  modified_base (34)..(39): a, c, t, g, unknown or other
tcgtcggcagcgtcagatgtgtataagagacagnnnnnngctgcagcttccttacacttcc

SEQ ID NO: 66 - DNA, 64 bp, Artificial Sequence
  source: /note="Description of Artificial Sequence: Synthetic primer"
  modified_base (35)..(40): a, c, t, g, unknown or other
gtctcgtgggctcggagatgtgtataagagacagnnnnnngaggaatatgtcccagatagcact

SEQ ID NO: 67 - DNA, 64 bp, Artificial Sequence
  source: /note="Description of Artificial Sequence: Synthetic primer"
  modified_base (34)..(39): a, c, t, g, unknown or other
tcgtcggcagcgtcagatgtgtataagagacagnnnnnnctgtgggatttcatggaagttcagc

SEQ ID NO: 68 - DNA, 59 bp, Artificial Sequence
  source: /note="Description of Artificial Sequence: Synthetic primer"
  modified_base (35)..(40): a, c, t, g, unknown or other
gtctcgtgggctcggagatgtgtataagagacagnnnnnnatcctggctggcaaggtgg

SEQ ID NO: 69 - DNA, 60 bp, Artificial Sequence
  source: /note="Description of Artificial Sequence: Synthetic primer"
  modified_base (34)..(39): a, c, t, g, unknown or other
tcgtcggcagcgtcagatgtgtataagagacagnnnnnnttccttggcctctgactgttg

SEQ ID NO: 70 - DNA, 61 bp, Artificial Sequence
  source: /note="Description of Artificial Sequence: Synthetic primer"
  modified_base (35)..(40): a, c, t, g, unknown or other
gtctcgtgggctcggagatgtgtataagagacagnnnnnnttcctgcccaccatctactcc

SEQ ID NO: 71 - DNA, 61 bp, Artificial Sequence
  source: /note="Description of Artificial Sequence: Synthetic primer"
  modified_base (34)..(39): a, c, t, g, unknown or other
tcgtcggcagcgtcagatgtgtataagagacagnnnnnngatgggcctcagtaccacattg

SEQ ID NO: 72 - DNA, 62 bp, Artificial Sequence
  source: /note="Description of Artificial Sequence: Synthetic primer"
  modified_base (35)..(40): a, c, t, g, unknown or other
gtctcgtgggctcggagatgtgtataagagacagnnnnnncaacctttgccttcccctaacc

SEQ ID NO: 73 - DNA, 23 bp, Homo sapiens
ggcactgcggctggaggtggggg

SEQ ID NO: 74 - DNA, 23 bp, Homo sapiens
ggcacgacggctggaggtggggg

SEQ ID NO: 75 - DNA, 23 bp, Homo sapiens
gctgcagaagggattccatgagg

SEQ ID NO: 76 - DNA, 23 bp, Homo sapiens
gctgcagaagggattccaagggg

SEQ ID NO: 77 - DNA, 23 bp, Homo sapiens
cacgttcaccttgccccacaggg

SEQ ID NO: 78 - DNA, 23 bp, Homo sapiens
cacgttcactttgccccacaggg

SEQ ID NO: 79 - DNA, 23 bp, Homo sapiens
ctccctcccaggatcctctctgg

SEQ ID NO: 80 - DNA, 23 bp, Homo sapiens
gccagtagccagccccgtcctgg

SEQ ID NO: 81 - DNA, 23 bp, Homo sapiens
caggcagtcttcatccccgtagg

SEQ ID NO: 82 - DNA, 23 bp, Homo sapiens
gaagcgtgatgacaaagaggagg

SEQ ID NO: 83 - DNA, 23 bp, Homo sapiens
attctggtcaacgtgtccttcgg